European Patent Application EP 4 732 851 A9, published June 3, 2026. Title: 一种连接子、抗体药物偶联物及其制备方法. Applicant: 复旦大学. The sequence listing filed with the application follows.

SEQUENCE LISTING (11 sequences)

SEQ ID NO: 1 - protein, 8 aa, synthetic construct
ETISSTYI

SEQ ID NO: 2 - protein, 8 aa, synthetic construct
ISGDGVTH

SEQ ID NO: 3 - protein, 8 aa, synthetic construct
YAAGRWNH

SEQ ID NO: 4 - protein, 114 aa, synthetic construct
QVQLVESGGGLVQPGGSLSLSCTASETISSTYIMGWHRRSPGKERELVAVISGDGVTHYADFVKGRFVISRDNAKNAVYLKMNFLTPEDTAVYYCYAAGRWNHWGQGTQVTVSS

SEQ ID NO: 5 - protein, 346 aa, synthetic construct
QVQLVESGGGLVQPGGSLSLSCTASETISSTYIMGWHRRSPGKERELVAVISGDGVTHYADFVKGRFVISRDNAKNAVYLKMNFLTPEDTAVYYCYAAGRWNHWGQGTQVTVSSEPKSSDKTHTCPPCPAPELLGGPSVFLFPPKPKDTLMISRTPEVTCVVVDVSHEDPEVKFNWYVDGVEVHNAKTKPREEQYNSTYRVVSVLTVLHQDWLNGKEYKCKVSNKALPAPIEKTISKAKGQPREPQVYTLPPSREEMTKNQVSLTCLVKGFYPSDIAVEWESNGQPENNYKTTPPVLDSDGSFFLYSKLTVDKSRWQQGNVFSCSVMHEALHNHYTQKSLSLSPGK

SEQ ID NO: 6 - protein, 346 aa, synthetic construct
QVQLVESGGGLVKPGGSLRLSCTASETISSTYIMGWHRQAPGKGRELVAVISGDGVTHYADFVKGRFTISRDNAKNTVYLQMNFLRAEDTAVYYCYAAGRWNHWGQGTMVTVSSEPKSSDKTHTCPPCPAPELLGGPSVFLFPPKPKDTLMISRTPEVTCVVVDVSHEDPEVKFNWYVDGVEVHNAKTKPREEQYNSTYRVVSVLTVLHQDWLNGKEYKCKVSNKALPAPIEKTISKAKGQPREPQVYTLPPSREEMTKNQVSLTCLVKGFYPSDIAVEWESNGQPENNYKTTPPVLDSDGSFFLYSKLTVDKSRWQQGNVFSCSVMHEALHNHYTQKSLSLSPGK

SEQ ID NO: 7 - protein, 357 aa, synthetic construct
QVQLVESGGGKAQPGGSLRLSCVASRITFRHYDLSWYRQAPGQERELVATVTNGGVITYADSVKGRFTISRDNAKNTVQLQMNNLKPEDTAVYYCNAVWVYLQRLTQNKKENDYWGPGTQVTVSSEPKSSDKTHTCPPCPAPELLGGPSVFLFPPKPKDTLMISRTPEVTCVVVDVSHEDPEVKFNWYVDGVEVHNAKTKPREEQYNSTYRVVSVLTVLHQDWLNGKEYKCKVSNKALPAPIEKTISKAKGQPREPQVYTLPPSREEMTKNQVSLTCLVKGFYPSDIAVEWESNGQPENNYKTTPPVLDSDGSFFLYSKLTVDKSRWQQGNVFSCSVMHEALHNHYTQKSLSLSPGK

SEQ ID NO: 8 - protein, 357 aa, synthetic construct
QVQLVESGGGLVQPGGSLRLSCSASRITFRHYDLSWYRQAPGKGRELVATVTNGGVITYADSVKGRFTISRDNAKNTVYLQMNNLRAEDTAVYYCNAVWVYLQRLTQNKKENDYWGQGTLVTVSSEPKSSDKTHTCPPCPAPELLGGPSVFLFPPKPKDTLMISRTPEVTCVVVDVSHEDPEVKFNWYVDGVEVHNAKTKPREEQYNSTYRVVSVLTVLHQDWLNGKEYKCKVSNKALPAPIEKTISKAKGQPREPQVYTLPPSREEMTKNQVSLTCLVKGFYPSDIAVEWESNGQPENNYKTTPPVLDSDGSFFLYSKLTVDKSRWQQGNVFSCSVMHEALHNHYTQKSLSLSPGK

SEQ ID NO: 9 - protein, 357 aa, synthetic construct
QVQLVESGGGLVKPGGSLRLSCAASRITFRHYDLSWYRQAPGKGRELVATVTNGGVITYADSVKGRFTISRDNAKNTVYLQMNNLRAEDTAVYYCNAVWVYLQRLTQNKKENDYWGQGTLVTVSSEPKSSDKTHTCPPCPAPELLGGPSVFLFPPKPKDTLMISRTPEVTCVVVDVSHEDPEVKFNWYVDGVEVHNAKTKPREEQYNSTYRVVSVLTVLHQDWLNGKEYKCKVSNKALPAPIEKTISKAKGQPREPQVYTLPPSREEMTKNQVSLTCLVKGFYPSDIAVEWESNGQPENNYKTTPPVLDSDGSFFLYSKLTVDKSRWQQGNVFSCSVMHEALHNHYTQKSLSLSPGK

SEQ ID NO: 10 - protein, 117 aa, synthetic construct
EVQLVQSGAEVKKPGESLKISCKGSGYSFTSYWMNWVRQMPGKGLEWMGMIYPADSETRLNQKFKDQATLSVDKSISTAYLQWSSLKASDTAMYYCAREDYGSSDYWGQGTTVTVSS

SEQ ID NO: 11 - protein, 106 aa, synthetic construct
DIQLTQSPSSLSASVGDRVTITCSASSSVSYMNWYQQKPGKSPKIWIYGISNLASGVPSRFSGSGSGTDFTLTISSLQPEDFATYYCQQKSSFPWTFGGGTKVEIK